European Patent Specification EP 4 289 960 B1, published July 15, 2026. Title: PREPARATION METHOD FOR MODIFIED TOXIN POLYPEPTIDE. Applicant: CHONGQING CLARUVIS PHARMACEUTICAL CO., LTD. The sequence listing filed with the application follows.

SEQUENCE LISTING (11 sequences)

SEQ ID NO: 1 - DNA, 654 bp, Artificial Sequence
atgtcccctatactaggttattggaaaattaagggccttgtgcaacccactcgacttcttttggaatatcttgaagaaaaatatgaagagcatttgtatgagcgcgatgaaggtgataaatggcgaaacaaaaagtttgaattgggtttggagtttcccaatcttccttattatattgatggtgatgttaaattaacacagtctatggccatcatacgttatatagctgacaagcacaacatgttgggtggttgtccaaaagagcgtgcagagatttcaatgcttgaaggagcggttttggatattagatacggtgtttcgagaattgcatatagtaaagactttgaaactctcaaagttgattttcttagcaagctacctgaaatgctgaaaatgttcgaagatcgtttatgtcataaaacatatttaaatggtgatcatgtaacccatcctgacttcatgttgtatgacgctcttgatgttgttttatacatggacccaatgtgcctggatgcgttcccaaaattagtttgttttaaaaaacgtattgaagctatcccacaaattgataagtacttgaaatccagcaagtatatagcatggcctttgcagggctggcaagccacgtttggtggtggcgaccatcctccaaaa

SEQ ID NO: 2 - protein, 218 aa, Artificial Sequence
MSPILGYWKIKGLVQPTRLLLEYLEEKYEEHLYERDEGDKWRNKKFELGLEFPNLPYYIDGDVKLTQSMAIIRYIADKHNMLGGCPKERAEISMLEGAVLDIRYGVSRIAYSKDFETLKVDFLSKLPEMLKMFEDRLCHKTYLNGDHVTHPDFMLYDALDVVLYMDPMCLDAFPKLVCFKKRIEAIPQIDKYLKSSKYIAWPLQGWQATFGGGDHPPK

SEQ ID NO: 3 - DNA, 24 bp, Artificial Sequence
ctggaagttctgttccaggggccc

SEQ ID NO: 4 - protein, 8 aa, Artificial Sequence
LEVLFQGP

SEQ ID NO: 5 - DNA, 6 bp, Artificial Sequence
ggatcc

SEQ ID NO: 6 - DNA, 3882 bp, Artificial Sequence
atgcctttcgttaacaaacagtttaactataaggacccggttaacggtgtggatattgcatacattaagatccctaacgctggtcagatgcagccggtgaaagcattcaagatccacaataagatttgggtgatcccggaacgcgatacctttaccaacccggaagaaggcgatctgaacccccctccggaggccaagcaagttcccgttagctattacgacagtacctatttaagcaccgataatgagaaagataactatctgaagggtgttaccaaactgttcgagcgcatctacagcacagacttaggccgcatgctgctgaccagtatcgttcgtggtattccgttctggggcggcagtaccatcgacaccgagctgaaagtgatcgacaccaattgcattaacgtgatccagcccgatggcagctatcgtagcgaagagctgaatctggttatcatcggccctagtgccgacattattcaattcgagtgtaaaagcttcggccatgaggtgctgaatttaacccgtaatggctatggcagtacccagtacatccgcttcagcccggattttaccttcggcttcgaggaatctttagaagtggataccaatccgctgctgggcgccggcaaatttgcaacagaccccgctgttactttagcccatgagctgattcatgctggtcatcgtctgtacggcatcgccattaacccgaaccgtgtgtttaaggttaacaccaacgcctattatgaaatgagtggtttagaggtgagcttcgaggagctgcgtacctttggtggccatgatgccaagttcatcgatagtctgcaagaaaacgagtttcgtctgtattattacaacaagttcaaagatatcgcaagcaccttaaataaagccaagagcatcgttggcaccaccgcctctttacaatatatgaaaaacgttttcaaggagaaatatctgctgagcgaggacaccagtggtaaatttagtgttgacaaactgaagttcgataaactgtataagatgctgaccgagatctataccgaagacaatttcgtgaaattttttaaagttctgaatcgcaaaacatatttaaacttcgacaaagcagtgtttaaaatcaacatcgttccgaaggttaattacacaatctacgatggcttcaatttacgcaacaccaatttagccgcaaacttcaacggccaaaataccgagatcaataacatgaatttcaccaaactgaaaaactttactggtttatttgagttctacaaactgctgtgcgtgcgtggcattatcaccagtttagaagtgctgtttcaaggtccggccttaaacgatctgtgtattaaagttaacaattgggatctgtttttcagccctagcgaggacaattttaccaacgatttaaacaaaggcgaggagatcaccagcgataccaatattgaggccgcagaggagaatatcagtctggatttaatccagcaatattatctgacctttaattttgacaatgagccggagaacattagtatcgaaaatttaagtagcgacatcattggtcagctggagctgatgccgaacattgagcgcttcccgaatggcaaaaagtatgaattagataagtacaccatgtttcactatttacgcgcccaagaatttgaacacggtaaaagccgtattgccttaaccaacagcgtgaatgaagcactgctgaacccgagccgcgtgtatacctttttcagtagtgactatgttaagaaggtgaataaggccaccgaagccgccatgttcttaggctgggtggagcagctggtgtatgatttcaccgatgagaccagcgaggtgagcaccacagataaaatcgcagatattacaattattattccgtacatcggcccggctttaaatatcggtaacatgctgtacaaagatgatttcgtgggcgctttaatctttagcggtgccgttattctgttagaattcattcccgaaattgcaatcccggtgctgggcacctttgctttagttagctatatcgcaaataaagtgttaaccgttcagaccattgacaatgctttaagcaagcgtaatgaaaagtgggatgaggtttataaatacatcgttacaaattggttagccaaagtgaacacccagattgatttaatccgtaagaaaatgaaagaagccttagagaatcaagctgaggccacaaaagcaattatcaattaccagtacaatcagtataccgaagaagaaaagaacaatatcaactttaatattgatgatttaagcagcaagctgaacgaaagcattaataaagccatgattaatattaacaagtttttaaaccagtgcagcgtgagctatttaatgaacagcatgatcccttacggtgtgaagcgtctggaagatttcgatgcctctttaaaagacgcactgttaaagtatatttatgacaatcgcggcacactgatcggtcaagttgatcgtctgaaagataaagttaataacacattaagcacagacattcctttccagctgagtaaatacgtggacaatcaacgtctgctgagcacctttaccgaatacattaaaaacattattaacaccagcattctgaatttacgctacgagagcaaccatttaattgatctgagccgttacgccagcaagatcaatatcggtagcaaggttaacttcgacccgattgacaaaaaccagatccagttattcaatttagagagtagtaagattgaggttattttaaaaaacgccatcgtttataacagcatgtacgaaaattttagcacaagcttttggattcgtatcccgaagtatttcaatagcatctctttaaataatgaatacacaatcattaattgcatggaaaacaacagcggctggaaggtgtctttaaactacggtgagatcatctggactttacaagatacccaagaaatcaagcagcgcgttgtgttcaaatatagtcagatgatcaacattagtgactatattaaccgctggatttttgtgaccatcacaaataaccgtttaaacaacagcaaaatttatattaacggtcgtctgattgaccagaagccgattagcaatttaggtaatatccatgccagcaacaacattatgttcaaactggatggttgtcgcgatacccatcgctacatctggattaagtactttaacttattcgacaaagaactgaatgaaaaggagatcaaggacttatatgataatcaaagcaatagcggcattttaaaagacttttggggtgactatctgcagtatgacaaaccttactatatgctgaacttatatgacccgaacaaatacgttgacgtgaacaatgtgggtattcgtggctacatgtatctgaaaggcccgcgcggcagtgttatgaccacaaatatttatttaaacagctctttatatcgtggcaccaagtttatcatcaagaagtacgcaagcggcaataaagacaatattgtgcgtaacaacgatcgtgtgtacatcaacgttgtggtgaagaacaaagagtatcgtttagccaccaatgccagccaagctggtgtggaaaaaattttaagcgcactggagatccccgatgtgggcaatttaagtcaagttgttgtgatgaaaagtaagaatgatcaaggcatcaccaacaaatgtaagatgaatttacaagacaataacggcaatgacattggttttattggtttccatcagttcaacaatatcgcaaagctggtggccagcaactggtacaaccgtcagatcgaacgtagcagccgtactttaggttgcagctgggaatttattccggtggatgatggttggggtgagcgccctttataa

SEQ ID NO: 7 - protein, 1293 aa, Artificial Sequence
MPFVNKQFNYKDPVNGVDIAYIKIPNAGQMQPVKAFKIHNKIWVIPERDTFTNPEEGDLNPPPEAKQVPVSYYDSTYLSTDNEKDNYLKGVTKLFERIYSTDLGRMLLTSIVRGIPFWGGSTIDTELKVIDTNCINVIQPDGSYRSEELNLVIIGPSADIIQFECKSFGHEVLNLTRNGYGSTQYIRFSPDFTFGFEESLEVDTNPLLGAGKFATDPAVTLAHELIHAGHRLYGIAINPNRVFKVNTNAYYEMSGLEVSFEELRTFGGHDAKFIDSLQENEFRLYYYNKFKDIASTLNKAKSIVGTTASLQYMKNVFKEKYLLSEDTSGKFSVDKLKFDKLYKMLTEIYTEDNFVKFFKVLNRKTYLNFDKAVFKINIVPKVNYTIYDGFNLRNTNLAANFNGQNTEINNMNFTKLKNFTGLFEFYKLLCVRGIITSLEVLFQGPALNDLCIKVNNWDLFFSPSEDNFTNDLNKGEEITSDTNIEAAEENISLDLIQQYYLTFNFDNEPENISIENLSSDIIGQLELMPNIERFPNGKKYELDKYTMFHYLRAQEFEHGKSRIALTNSVNEALLNPSRVYTFFSSDYVKKVNKATEAAMFLGWVEQLVYDFTDETSEVSTTDKIADITIIIPYIGPALNIGNMLYKDDFVGALIFSGAVILLEFIPEIAIPVLGTFALVSYIANKVLTVQTIDNALSKRNEKWDEVYKYIVTNWLAKVNTQIDLIRKKMKEALENQAEATKAIINYQYNQYTEEEKNNINFNIDDLSSKLNESINKAMININKFLNQCSVSYLMNSMIPYGVKRLEDFDASLKDALLKYIYDNRGTLIGQVDRLKDKVNNTLSTDIPFQLSKYVDNQRLLSTFTEYIKNIINTSILNLRYESNHLIDLSRYASKINIGSKVNFDPIDKNQIQLFNLESSKIEVILKNAIVYNSMYENFSTSFWIRIPKYFNSISLNNEYTIINCMENNSGWKVSLNYGEIIWTLQDTQEIKQRVVFKYSQMINISDYINRWIFVTITNNRLNNSKIYINGRLIDQKPISNLGNIHASNNIMFKLDGCRDTHRYIWIKYFNLFDKELNEKEIKDLYDNQSNSGILKDFWGDYLQYDKPYYMLNLYDPNKYVDVNNVGIRGYMYLKGPRGSVMTTNIYLNSSLYRGTKFIIKKYASGNKDNIVRNNDRVYINVVVKNKEYRLATNASQAGVEKILSALEIPDVGNLSQVVVMKSKNDQGITNKCKMNLQDNNGNDIGFIGFHQFNNIAKLVASNWYNRQIERSSRTLGCSWEFIPVDDGWGERPL

SEQ ID NO: 8 - DNA, 24 bp, Artificial Sequence
ttagaagtgctgtttcaaggtccg

SEQ ID NO: 9 - protein, 8 aa, Artificial Sequence
LEVLFQGP

SEQ ID NO: 10 - DNA, 4575 bp, Artificial Sequence
atgtcccctatactaggttattggaaaattaagggccttgtgcaacccactcgacttcttttggaatatcttgaagaaaaatatgaagagcatttgtatgagcgcgatgaaggtgataaatggcgaaacaaaaagtttgaattgggtttggagtttcccaatcttccttattatattgatggtgatgttaaattaacacagtctatggccatcatacgttatatagctgacaagcacaacatgttgggtggttgtccaaaagagcgtgcagagatttcaatgcttgaaggagcggttttggatattagatacggtgtttcgagaattgcatatagtaaagactttgaaactctcaaagttgattttcttagcaagctacctgaaatgctgaaaatgttcgaagatcgtttatgtcataaaacatatttaaatggtgatcatgtaacccatcctgacttcatgttgtatgacgctcttgatgttgttttatacatggacccaatgtgcctggatgcgttcccaaaattagtttgttttaaaaaacgtattgaagctatcccacaaattgataagtacttgaaatccagcaagtatatagcatggcctttgcagggctggcaagccacgtttggtggtggcgaccatcctccaaaatcggatctggaagttctgttccaggggcccctgggatccatgcctttcgttaacaaacagtttaactataaggacccggttaacggtgtggatattgcatacattaagatccctaacgctggtcagatgcagccggtgaaagcattcaagatccacaataagatttgggtgatcccggaacgcgatacctttaccaacccggaagaaggcgatctgaacccccctccggaggccaagcaagttcccgttagctattacgacagtacctatttaagcaccgataatgagaaagataactatctgaagggtgttaccaaactgttcgagcgcatctacagcacagacttaggccgcatgctgctgaccagtatcgttcgtggtattccgttctggggcggcagtaccatcgacaccgagctgaaagtgatcgacaccaattgcattaacgtgatccagcccgatggcagctatcgtagcgaagagctgaatctggttatcatcggccctagtgccgacattattcaattcgagtgtaaaagcttcggccatgaggtgctgaatttaacccgtaatggctatggcagtacccagtacatccgcttcagcccggattttaccttcggcttcgaggaatctttagaagtggataccaatccgctgctgggcgccggcaaatttgcaacagaccccgctgttactttagcccatgagctgattcatgctggtcatcgtctgtacggcatcgccattaacccgaaccgtgtgtttaaggttaacaccaacgcctattatgaaatgagtggtttagaggtgagcttcgaggagctgcgtacctttggtggccatgatgccaagttcatcgatagtctgcaagaaaacgagtttcgtctgtattattacaacaagttcaaagatatcgcaagcaccttaaataaagccaagagcatcgttggcaccaccgcctctttacaatatatgaaaaacgttttcaaggagaaatatctgctgagcgaggacaccagtggtaaatttagtgttgacaaactgaagttcgataaactgtataagatgctgaccgagatctataccgaagacaatttcgtgaaattttttaaagttctgaatcgcaaaacatatttaaacttcgacaaagcagtgtttaaaatcaacatcgttccgaaggttaattacacaatctacgatggcttcaatttacgcaacaccaatttagccgcaaacttcaacggccaaaataccgagatcaataacatgaatttcaccaaactgaaaaactttactggtttatttgagttctacaaactgctgtgcgtgcgtggcattatcaccagtttagaagtgctgtttcaaggtccggccttaaacgatctgtgtattaaagttaacaattgggatctgtttttcagccctagcgaggacaattttaccaacgatttaaacaaaggcgaggagatcaccagcgataccaatattgaggccgcagaggagaatatcagtctggatttaatccagcaatattatctgacctttaattttgacaatgagccggagaacattagtatcgaaaatttaagtagcgacatcattggtcagctggagctgatgccgaacattgagcgcttcccgaatggcaaaaagtatgaattagataagtacaccatgtttcactatttacgcgcccaagaatttgaacacggtaaaagccgtattgccttaaccaacagcgtgaatgaagcactgctgaacccgagccgcgtgtatacctttttcagtagtgactatgttaagaaggtgaataaggccaccgaagccgccatgttcttaggctgggtggagcagctggtgtatgatttcaccgatgagaccagcgaggtgagcaccacagataaaatcgcagatattacaattattattccgtacatcggcccggctttaaatatcggtaacatgctgtacaaagatgatttcgtgggcgctttaatctttagcggtgccgttattctgttagaattcattcccgaaattgcaatcccggtgctgggcacctttgctttagttagctatatcgcaaataaagtgttaaccgttcagaccattgacaatgctttaagcaagcgtaatgaaaagtgggatgaggtttataaatacatcgttacaaattggttagccaaagtgaacacccagattgatttaatccgtaagaaaatgaaagaagccttagagaatcaagctgaggccacaaaagcaattatcaattaccagtacaatcagtataccgaagaagaaaagaacaatatcaactttaatattgatgatttaagcagcaagctgaacgaaagcattaataaagccatgattaatattaacaagtttttaaaccagtgcagcgtgagctatttaatgaacagcatgatcccttacggtgtgaagcgtctggaagatttcgatgcctctttaaaagacgcactgttaaagtatatttatgacaatcgcggcacactgatcggtcaagttgatcgtctgaaagataaagttaataacacattaagcacagacattcctttccagctgagtaaatacgtggacaatcaacgtctgctgagcacctttaccgaatacattaaaaacattattaacaccagcattctgaatttacgctacgagagcaaccatttaattgatctgagccgttacgccagcaagatcaatatcggtagcaaggttaacttcgacccgattgacaaaaaccagatccagttattcaatttagagagtagtaagattgaggttattttaaaaaacgccatcgtttataacagcatgtacgaaaattttagcacaagcttttggattcgtatcccgaagtatttcaatagcatctctttaaataatgaatacacaatcattaattgcatggaaaacaacagcggctggaaggtgtctttaaactacggtgagatcatctggactttacaagatacccaagaaatcaagcagcgcgttgtgttcaaatatagtcagatgatcaacattagtgactatattaaccgctggatttttgtgaccatcacaaataaccgtttaaacaacagcaaaatttatattaacggtcgtctgattgaccagaagccgattagcaatttaggtaatatccatgccagcaacaacattatgttcaaactggatggttgtcgcgatacccatcgctacatctggattaagtactttaacttattcgacaaagaactgaatgaaaaggagatcaaggacttatatgataatcaaagcaatagcggcattttaaaagacttttggggtgactatctgcagtatgacaaaccttactatatgctgaacttatatgacccgaacaaatacgttgacgtgaacaatgtgggtattcgtggctacatgtatctgaaaggcccgcgcggcagtgttatgaccacaaatatttatttaaacagctctttatatcgtggcaccaagtttatcatcaagaagtacgcaagcggcaataaagacaatattgtgcgtaacaacgatcgtgtgtacatcaacgttgtggtgaagaacaaagagtatcgtttagccaccaatgccagccaagctggtgtggaaaaaattttaagcgcactggagatccccgatgtgggcaatttaagtcaagttgttgtgatgaaaagtaagaatgatcaaggcatcaccaacaaatgtaagatgaatttacaagacaataacggcaatgacattggttttattggtttccatcagttcaacaatatcgcaaagctggtggccagcaactggtacaaccgtcagatcgaacgtagcagccgtactttaggttgcagctgggaatttattccggtggatgatggttggggtgagcgccctttataa

SEQ ID NO: 11 - protein, 1524 aa, Artificial Sequence
MSPILGYWKIKGLVQPTRLLLEYLEEKYEEHLYERDEGDKWRNKKFELGLEFPNLPYYIDGDVKLTQSMAIIRYIADKHNMLGGCPKERAEISMLEGAVLDIRYGVSRIAYSKDFETLKVDFLSKLPEMLKMFEDRLCHKTYLNGDHVTHPDFMLYDALDVVLYMDPMCLDAFPKLVCFKKRIEAIPQIDKYLKSSKYIAWPLQGWQATFGGGDHPPKSDLEVLFQGPLGSMPFVNKQFNYKDPVNGVDIAYIKIPNAGQMQPVKAFKIHNKIWVIPERDTFTNPEEGDLNPPPEAKQVPVSYYDSTYLSTDNEKDNYLKGVTKLFERIYSTDLGRMLLTSIVRGIPFWGGSTIDTELKVIDTNCINVIQPDGSYRSEELNLVIIGPSADIIQFECKSFGHEVLNLTRNGYGSTQYIRFSPDFTFGFEESLEVDTNPLLGAGKFATDPAVTLAHELIHAGHRLYGIAINPNRVFKVNTNAYYEMSGLEVSFEELRTFGGHDAKFIDSLQENEFRLYYYNKFKDIASTLNKAKSIVGTTASLQYMKNVFKEKYLLSEDTSGKFSVDKLKFDKLYKMLTEIYTEDNFVKFFKVLNRKTYLNFDKAVFKINIVPKVNYTIYDGFNLRNTNLAANFNGQNTEINNMNFTKLKNFTGLFEFYKLLCVRGIITSLEVLFQGPALNDLCIKVNNWDLFFSPSEDNFTNDLNKGEEITSDTNIEAAEENISLDLIQQYYLTFNFDNEPENISIENLSSDIIGQLELMPNIERFPNGKKYELDKYTMFHYLRAQEFEHGKSRIALTNSVNEALLNPSRVYTFFSSDYVKKVNKATEAAMFLGWVEQLVYDFTDETSEVSTTDKIADITIIIPYIGPALNIGNMLYKDDFVGALIFSGAVILLEFIPEIAIPVLGTFALVSYIANKVLTVQTIDNALSKRNEKWDEVYKYIVTNWLAKVNTQIDLIRKKMKEALENQAEATKAIINYQYNQYTEEEKNNINFNIDDLSSKLNESINKAMININKFLNQCSVSYLMNSMIPYGVKRLEDFDASLKDALLKYIYDNRGTLIGQVDRLKDKVNNTLSTDIPFQLSKYVDNQRLLSTFTEYIKNIINTSILNLRYESNHLIDLSRYASKINIGSKVNFDPIDKNQIQLFNLESSKIEVILKNAIVYNSMYENFSTSFWIRIPKYFNSISLNNEYTIINCMENNSGWKVSLNYGEIIWTLQDTQEIKQRVVFKYSQMINISDYINRWIFVTITNNRLNNSKIYINGRLIDQKPISNLGNIHASNNIMFKLDGCRDTHRYIWIKYFNLFDKELNEKEIKDLYDNQSNSGILKDFWGDYLQYDKPYYMLNLYDPNKYVDVNNVGIRGYMYLKGPRGSVMTTNIYLNSSLYRGTKFIIKKYASGNKDNIVRNNDRVYINVVVKNKEYRLATNASQAGVEKILSALEIPDVGNLSQVVVMKSKNDQGITNKCKMNLQDNNGNDIGFIGFHQFNNIAKLVASNWYNRQIERSSRTLGCSWEFIPVDDGWGERPL